European Patent Application EP 4 279 500 A1, published November 22, 2023. Title: Compound or salt thereof or antibody obtained thereby. Applicant: Ajinomoto Co., Inc. The sequence listing filed with the application follows.

SEQUENCE LISTING (11 sequences)

SEQ ID NO: 1 - protein, 30 aa, Artificial Sequence
  Affinity peptide capable of binding to CH2 domain of immunoglobulin unit
CQRRFYEALHDPNLNEEQRNARIRSIKDDC

SEQ ID NO: 2 - protein, 34 aa, Artificial Sequence
  Affinity peptide capable of binding to CH2 domain of immunoglobulin unit
FNMQCQRRFYEALHDPNLNEEQRNARIRSIKDDC

SEQ ID NO: 3 - protein, 34 aa, Artificial Sequence
  Affinity peptide capable of binding to CH2 domain of immunoglobulin unit
FNMQCQRRFYEALHDPNLNEEQRNARIRSIKEDC

SEQ ID NO: 4 - protein, 34 aa, Artificial Sequence
  Affinity peptide capable of binding to CH2 domain of immunoglobulin unit
FNMQCQRRFYEALHDPNLNEEQRNARIRSIKEEC

SEQ ID NO: 5 - protein, 33 aa, Artificial Sequence
  Affinity peptide capable of binding to CH2 domain of immunoglobulin unit
NMQCQRRFYEALHDPNLNEEQRNARIRSIKEEC

SEQ ID NO: 6 - protein, 32 aa, Artificial Sequence
  Affinity peptide capable of binding to CH2 domain of immunoglobulin unit
MQCQRRFYEALHDPNLNEEQRNARIRSIKEEC

SEQ ID NO: 7 - protein, 31 aa, Artificial Sequence
  Affinity peptide capable of binding to CH2 domain of immunoglobulin unit
QCQRRFYEALHDPNLNEEQRNARIRSIKEEC

SEQ ID NO: 8 - protein, 449 aa, Artificial Sequence
  Amino acid sequence of heavy chain in trastuzumab
EVQLVESGGGLVQPGGSLRLSCAASGFNIKDTYIHWVRQAPGKGLEWVARIYPTNGYTRYADSVKGRFTISADTSKNTAYLQMNSLRAEDTAVYYCSRWGGDGFYAMDYWGQGTLVTVSSASTKGPSVFPLAPSSKSTSGGTAALGCLVKDYFPEPVTVSWNSGALTSGVHTFPAVLQSSGLYSLSSVVTVPSSSLGTQTYICNVNHKPSNTKVDKKVEPKSCDKTHTCPPCPAPELLGGPSVFLFPPKPKDTLMISRTPEVTCVVVDVSHEDPEVKFNWYVDGVEVHNAKTKPREEQYDSTYRVVSVLTVLHQDWLNGKEYKCKVSNKALPAPIEKTISKAKGQPREPQVYTLPPSREEMTKNQVSLTCLVKGFYPSDIAVEWESNGQPENNYKTTPPVLDSDGSFFLYSKLTVDKSRWQQGNVFSCSVMHEALHNHYTQKSLSLSPG

SEQ ID NO: 9 - protein, 214 aa, Artificial Sequence
  Amino acid sequence of light chain in trastuzumab
DIQMTQSPSSLSASVGDRVTITCRASQDVNTAVAWYQQKPGKAPKLLIYSASFLYSGVPSRFSGSRSGTDFTLTISSLQPEDFATYYCQQHYTTPPTFGQGTKVEIKRTVAAPSVFIFPPSDEQLKSGTASVVCLLNNFYPREAKVQWKVDNALQSGNSQESVTEQDSKDSTYSLSSTLTLSKADYEKHKVYACEVTHQGLSSPVTKSFNRGEC

SEQ ID NO: 10 - protein, 18 aa, Artificial Sequence
  Amino acid sequence of peptide fragment  obtained by cleaving trastuzumab with trypsin
FNWYVDGVEVHNAKTKPR

SEQ ID NO: 11 - protein, 17 aa, Artificial Sequence
  Affinity peptide capable of binding to CH2 domain of immunoglobulin unit
RGNCAYHKGQIIWCTYH